European Patent Application EP 4 450 518 A1, published October 23, 2024. Title: ＶＨＨ抗体. Applicant: 学校法人帝京平成大学. The sequence listing filed with the application follows.

SEQUENCE LISTING (15 sequences)

SEQ ID NO: 1 - protein, 5 aa, synthetic construct
  source 1..5: note = Designed peptide
NYAMG

SEQ ID NO: 2 - protein, 22 aa, synthetic construct
  source 1..22: note = Designed peptide
AIGWTTGTASYGTPTYSDSVKG

SEQ ID NO: 3 - protein, 18 aa, synthetic construct
  source 1..18: note = Designed peptide
GLIGYFGDRISSASVYDG

SEQ ID NO: 4 - protein, 132 aa, synthetic construct
EVQLVESGGGLVQAGNSLKLSCVVSGRTLRNYAMGWFRQAPLKEREFVAAIGWTTGTASYGTPTYSDSVKGRFTISRDNAGNTLYLLMNNLKPEDTAVYYCAAGLIGYFGDRISSASVYDGWGQGTQVTVSS

SEQ ID NO: 5 - protein, 5 aa, synthetic construct
  source 1..5: note = Designed peptide
GYAMK

SEQ ID NO: 6 - protein, 17 aa, synthetic construct
  source 1..17: note = Designed peptide
AIASDGGLTNYADFVKG

SEQ ID NO: 7 - protein, 9 aa, synthetic construct
  source 1..9: note = Designed peptide
VRGYSNSNY

SEQ ID NO: 8 - protein, 118 aa, synthetic construct
EVQLVESGGGLVQPGGSLKLSCAASGFTFNGYAMKWYRQAPGKGREFIAAIASDGGLTNYADFVKGRFTISRDNIINMVFLQMNSLKPEDTAVYFCNAVRGYSNSNYWGQGTQVTVSS

SEQ ID NO: 9 - protein, 132 aa, synthetic construct
EVQLLESGGGLVQAGNSLRLSCVVSGRTLRNYAMGWFRQAPLKEREFVAAIGWTTGTASYGTPTYSDSVKGRFTISRDNSKNTLYLLMNNLRPEDTAVYYCAAGLIGYFGDRISSASVYDGWGQGTLVTVSS

SEQ ID NO: 10 - protein, 118 aa, synthetic construct
EVQLLESGGGLVQPGGSLRLSCAASGFTFNGYAMKWYRQAPGKGREFIAAIASDGGLTNYADFVKGRFTISRDNSKNTVYLQMNSLRPEDTAVYYCNAVRGYSNSNYWGQGTLVTVSS

SEQ ID NO: 11 - DNA, 19 bp, synthetic construct
  source 1..19: mol_type = other DNA
ggtggtcctggctgctctt

SEQ ID NO: 12 - DNA, 19 bp, synthetic construct
  source 1..19: mol_type = other DNA
aggagacggtgacctgggt

SEQ ID NO: 13 - DNA, 49 bp, synthetic construct
  source 1..49: mol_type = other DNA
ggtaaaggcccagccggccatggccgaggtgcagctcgtggagtctggg

SEQ ID NO: 14 - DNA, 41 bp, synthetic construct
  source 1..41: mol_type = other DNA
ttgcaagcaattgcggccgctgaggagacggtgacctgggt

SEQ ID NO: 15 - protein, 485 aa, synthetic construct
  source 1..485: note = Designed peptide
MKRSFLSLAVAAVVLSGCSLIPDYQRPEAPVAAAYPQGQAYGQNTGAAAVPAADIGWREFFRDPQLQQLIGVALENNRDLRVAALNVEAFRAQYRIQRADLFPRIGVDGSGTRQRLPGDLSTTGSPAISSQYGVTLGTTAWELDLFGRLRSLRDQALEQYLATEQAQRSAQTTLVASVATAYLTLKADQAQLQLTKDTLGTYQKSFDLTQRSYDVGVASALDLRQAQTAVEGARATLAQYTRLVAQDQNALVLLLGSGIPANLPQGLGLDQTLLTEVPAGLPSDLLQRRPDILEAEHQLMAANASIGAARAAFFPSISLTANAGTMSRQLSGLFDAGSGSWLFQPSINLPIFTAGSLRASLDYAKIQKDINVAQYEKAIQTAFQEVADGLAARGTFTEQLQAQRDLVKASDEYYQLADKRYRTGVDNYLTLLDAQRSLFTAQQQLITDRLNQLTSEVNLYKALGGGWNQQTVTQQQTAKKEDPQA